European Patent Application EP 4 324 912 A1, published February 21, 2024. Title: Nutrient-rich stevia plant. Applicant: SUNTORY HOLDINGS LIMITED. The sequence listing filed with the application follows.

SEQUENCE LISTING (30 sequences)

SEQ ID NO: 1 - DNA, 70 bp, Stevia rebaudiana
ataaactttaggcccgacgatgttactctacacattycccgtcttgttcatggccgtagtgggaagtgta

SEQ ID NO: 2 - DNA, 23 bp, Stevia rebaudiana
ataaactttaggcccgacgatgt

SEQ ID NO: 3 - DNA, 20 bp, Stevia rebaudiana
tacacttcccactacggcca

SEQ ID NO: 4 - DNA, 21 bp, Stevia rebaudiana
tctacacattccccgtcttgt

SEQ ID NO: 5 - DNA, 41 bp, Stevia rebaudiana
acgatgttactctacacattccccgtcttgttcatggccgt

SEQ ID NO: 6 - DNA, 61 bp, Stevia rebaudiana
tttaggcccgacgatgttactctacacattccccgtcttgttcatggccgtagtgggaagt

SEQ ID NO: 7 - DNA, 38 bp, Artificial Sequence
  Synthetic DNA
gtataaactttaggcccgacgatgttactctacacatg

SEQ ID NO: 8 - DNA, 30 bp, Artificial Sequence
  Synthetic DNA
gagaaaggaaagatatatttaaccatcatg

SEQ ID NO: 9 - DNA, 220 bp, Artificial Sequence
  Synthetic DNA
gtataaactttaggcccgacgatgttactctacacatgccccgtcttgttcatggccgtagtgggaagtgtatatctccatttaagaaaaaaggcgaatcaaaaccgagatgaagggtatatatatatataatagttttttacttatttcagtaaattaaataactgtttatttttactttatactatttcatgatggttaaatatatctttcctttctc

SEQ ID NO: 10 - DNA, 220 bp, Artificial Sequence
  Synthetic DNA
gtataaactttaggcccgacgatgttactctacacatgtcccgtcttgttcatggccgtagtgggaagtgtatatctccatttaagaaaaaaggcgaatcaaaaccgagatgaagggtatatatatatataatagttttttacttatttcagtaaattaaataactgtttatttttactttatactatttcatgatggttaaatatatctttcctttctc

SEQ ID NO: 11 - DNA, 34 bp, Artificial Sequence
  Synthetic DNA
gtataaactttaggcccgacgatgttactctaca

SEQ ID NO: 12 - DNA, 186 bp, Artificial Sequence
  Synthetic DNA
catgtcccgtcttgttcatggccgtagtgggaagtgtatatctccatttaagaaaaaaggcgaatcaaaaccgagatgaagggtatatatatatataatagttttttacttatttcagtaaattaaataactgtttatttttactttatactatttcatgatggttaaatatatctttcctttctc

SEQ ID NO: 13 - DNA, 3232 bp, Stevia rebaudiana
atgattatgaagatgatcaaagggtttgcaattttgttgtttataggctaccttttcctatgggtgatcacaccaacctatgtattcaagcagaagtggctcgtgacggttcgagcccacaccacttctacttactttggaactcaaggtttgttccacctctccaatcaacattttttaaatcactctgatttactagtctaattacatcataatatatacaaaacataaaataacagatttaatagttttgttttctaactattttacgttttcttttaaatgtgtataaactttaggcccgacgatgttactctacacattycccgtcttgttcatggccgtagtgggaagtgtatatctccatttaagaaaaaaggcgaatcaaaaccgagatgaagggtatatatatatataatagttttttacttatttcagtaaattaaataactgtttatttttactttatactatttcatgatggttaaatatatctttcctttctcaaattttagagaaaaagaagctacacccgataacttgagtatatggagaagaccaatgatcatcaaaggtctcgggatcgtctcgaaaatcgagctcgctttctttgttatgtttatcgctcttatcgtctggtctttcacgacatacttacacgtcggttttgccaaaatcaatcataaaacagcggcaaaaaagggagaggaagtgtaagtgaatcaatattttaaatattttgcaaatactacattcgtatattattattaacccgcgatcgattcttttggttgatagttgggaatcaaagcttgattcggtggctctacggttcggattaattggcaacttgtgtctagcatttctgttcttcccggtgactcgaggatcgtctatattgtcgttgttcgggcttacttctgaggcgagtatcaagtatcacatatggctcggtcatattgttatgactctattcacttctcatggtgtttgttacattatttattggatcgttaccaaacagacacatgaggtaccttaatttttatattattatttatgaattataaattagttaatatttatggctcacaattcctgaaaatattctgccagtgaatttggaaaactgaagataaagtccataaatgttagaagattttccactttgaattaaagtcaacttatataatggtcccaaatcatcgaacattgtaaaaattaactcaccaatgtgaaaaaccgaagataggatcatatcccataactttattctttggtgatgaaatgacgaagctaacataatttatttaacagtcccttttaaaaatttctgatagatgttagacgtaattaattagttaattaattattactcaccgaacaatgacaaatgcttataaaagttgtttttgaactatcgttgttgatccgttgatgtcttttttcatatatgatatccaattttcctagtagtgtattaaataatgctatatgtttttttagatgttgaaatgggaaaaaatcggcatatcaaatgtagccggagagttggctttggtagccggattgattatgtgggcaacaacgtttccaaggattagacgaaagatgtttgaagttttcttctacgcacatcacttatacatccaatttatcgtgttcttcgtgttccatgttggcatagcatatgcatccatcatgctaccgggattctacctcttcatgattgatcgaatcttgagatttttacaatcaaagggaaacgttcgtgtggtttctgctcgtgttcttccgtgtgaatctctcgagctcaacttctccaaaagccaaggtacgtaaaatagagcacaaaaagtatagaaaatataaaggatcaatttctttttaagtgataatggtcgttaacatttgtcttttaattttaagtcttttagatgtcacaattttcatttttttatataggtctacaatatacaccaacaagcatcatattcatcaatgtcccaagcatttcaaaggctcaatggcatccattcaccattacttctagtagcaatttggagcccgaaaagctaagtgttatgatcaaaagtgaaggaagttggtctaggaaactttaccaaatgttatcatccccaaattctattgaccggcttgatgtatgcattgaaggaccttatgggcctatttcaaccaactttctaaggtattatgttcattacaatgacttgtgttaggttcatttcattttattatacttaaaatgatcaaattatggtttcaggcacgatatgctagtgatggtgagcggaggaagtgggataacaccatttatctcaatatttagggagcttgtttacactaccgaaaccctaaaacgtaaagctccaaaaattctcttgataagttcgtttaaagactcttctgatctcaccatgctagaattgttattaccatcatctggtgcacctatagagttttcaaaactagagttacaaatcgaggcatatgtgacaagagaaaaccagcccgttaatgataagaaactagtgactgccttatggtttaaaccaaatccctctgacgcacccatcactcctattttaggacaaaatggttggttatggcttggtgcgattattgcatgttcttttgtgattttccttgtatctatggggcttgtaacacggttttacatctatcctattgataataacaccaacaaggtgtattcatatggatcgagggccgtgttaaacatgttgctcatttgtgtgtctataatggtaacatgttgtttcggattttggtggaataaaaagagaaacgctatggactcaaagcaaattcaaagcatggagggtgtgacacccgttagctcacccaactcatggttttataacgcggatagagagcttgaaagtgttccccaacaatcgctctttcagtctacaaatgttcattttggcaaaagaccggatcttaagagtaagaccagattctatgtctaatgctacaaaagttacacacttttgaatatatgttaatacaaaccctaacactttctattttgtttatatttttgttaggaattttgtttgagcaaaaagaatcaagtgttggagttcttgtttgtgggccaaaaaagatgaggcatgaggctgcaaatatatgttcatccggattggcttcaaacttgcattttgagtccataagttttagttggtga

SEQ ID NO: 14 - DNA, 2097 bp, Stevia rebaudiana
  CDS (1)..(2097)
atgaagatgatcaaagggtttgcaattttgttgtttataggctaccttttcctatgggtgatcacaccaacctatgtattcaagcagaagtggctcgtgacggttcgagcccacaccacttctacttactttggaactcaaggtggcccgacgatgttactctacacattycccgtcttgttcatggccgtagtgggaagtgtatatctccatttaagaaaaaaggcgaatcaaaaccgagatgaagggaattttagagaaaaagaagctacacccgataacttgagtatatggagaagaccaatgatcatcaaaggtctcgggatcgtctcgaaaatcgagctcgctttctttgttatgtttatcgctcttatcgtctggtctttcacgacatacttacacgtcggttttgccaaaatcaatcataaaacagcggcaaaaaagggagaggaagtgtgggaatcaaagcttgattcggtggctctacggttcggattaattggcaacttgtgtctagcatttctgttcttcccggtgactcgaggatcgtctatattgtcgttgttcgggcttacttctgaggcgagtatcaagtatcacatatggctcggtcatattgttatgactctattcacttctcatggtgtttgttacattatttattggatcgttaccaaacagacacatgaggtaatgttgaaatgggaaaaaatcggcatatcaaatgtagccggagagttggctttggtagccggattgattatgtgggcaacaacgtttccaaggattagacgaaagatgtttgaagttttcttctacgcacatcacttatacatccaatttatcgtgttcttcgtgttccatgttggcatagcatatgcatccatcatgctaccgggattctacctcttcatgattgatcgaatcttgagatttttacaatcaaagggaaacgttcgtgtggtttctgctcgtgttcttccgtgtgaatctctcgagctcaacttctccaaaagccaaggtggtctacaatatacaccaacaagcatcatattcatcaatgtcccaagcatttcaaaggctcaatggcatccattcaccattacttctagtagcaatttggagcccgaaaagctaagtgttatgatcaaaagtgaaggaagttggtctaggaaactttaccaaatgttatcatccccaaattctattgaccggcttgatgtatgcattgaaggaccttatgggcctatttcaaccaactttctaaggcacgatatgctagtgatggtgagcggaggaagtgggataacaccatttatctcaatatttagggagcttgtttacactaccgaaaccctaaaacgtaaagctccaaaaattctcttgataagttcgtttaaagactcttctgatctcaccatgctagaattgttattaccatcatctggtgcacctatagagttttcaaaactagagttacaaatcgaggcatatgtgacaagagaaaaccagcccgttaatgataagaaactagtgactgccttatggtttaaaccaaatccctctgacgcacccatcactcctattttaggacaaaatggttggttatggcttggtgcgattattgcatgttcttttgtgattttccttgtatctatggggcttgtaacacggttttacatctatcctattgataataacaccaacaaggtgtattcatatggatcgagggccgtgttaaacatgttgctcatttgtgtgtctataatggtaacatgttgtttcggattttggtggaataaaaagagaaacgctatggactcaaagcaaattcaaagcatggagggtgtgacacccgttagctcacccaactcatggttttataacgcggatagagagcttgaaagtgttccccaacaatcgctctttcagtctacaaatgttcattttggcaaaagaccggatcttaaggagcaaaaagaatcaagtgttggagttcttgtttgtgggccaaaaaagatgaggcatgaggctgcaaatatatgttcatccggattggcttcaaacttgcattttgagtccataagttttagttgg

SEQ ID NO: 15 - protein, 699 aa, Stevia rebaudiana
MKMIKGFAILLFIGYLFLWVITPTYVFKQKWLVTVRAHTTSTYFGTQGGPTMLLYTFPVLFMAVVGSVYLHLRKKANQNRDEGNFREKEATPDNLSIWRRPMIIKGLGIVSKIELAFFVMFIALIVWSFTTYLHVGFAKINHKTAAKKGEEVWESKLDSVALRFGLIGNLCLAFLFFPVTRGSSILSLFGLTSEASIKYHIWLGHIVMTLFTSHGVCYIIYWIVTKQTHEVMLKWEKIGISNVAGELALVAGLIMWATTFPRIRRKMFEVFFYAHHLYIQFIVFFVFHVGIAYASIMLPGFYLFMIDRILRFLQSKGNVRVVSARVLPCESLELNFSKSQGGLQYTPTSIIFINVPSISKAQWHPFTITSSSNLEPEKLSVMIKSEGSWSRKLYQMLSSPNSIDRLDVCIEGPYGPISTNFLRHDMLVMVSGGSGITPFISIFRELVYTTETLKRKAPKILLISSFKDSSDLTMLELLLPSSGAPIEFSKLELQIEAYVTRENQPVNDKKLVTALWFKPNPSDAPITPILGQNGWLWLGAIIACSFVIFLVSMGLVTRFYIYPIDNNTNKVYSYGSRAVLNMLLICVSIMVTCCFGFWWNKKRNAMDSKQIQSMEGVTPVSSPNSWFYNADRELESVPQQSLFQSTNVHFGKRPDLKEQKESSVGVLVCGPKKMRHEAANICSSGLASNLHFESISFSW

SEQ ID NO: 16 - DNA, 21 bp, Stevia rebaudiana
tctacacatttcccgtcttgt

SEQ ID NO: 17 - DNA, 41 bp, Stevia rebaudiana
acgatgttactctacacatttcccgtcttgttcatggccgt

SEQ ID NO: 18 - DNA, 61 bp, Stevia rebaudiana
tttaggcccgacgatgttactctacacatttcccgtcttgttcatggccgtagtgggaagt

SEQ ID NO: 19 - DNA, 20 bp, Artificial Sequence
  Synthetic DNA
acgatgttactctacacatg

SEQ ID NO: 20 - DNA, 20 bp, Artificial Sequence
  Synthetic DNA
agatatatttaaccatcatg

SEQ ID NO: 21 - DNA, 70 bp, Stevia rebaudiana
ataaactttaggcccgacgatgttactctacacattccccgtcttgttcatggccgtagtgggaagtgta

SEQ ID NO: 22 - DNA, 3232 bp, Stevia rebaudiana
atgattatgaagatgatcaaagggtttgcaattttgttgtttataggctaccttttcctatgggtgatcacaccaacctatgtattcaagcagaagtggctcgtgacggttcgagcccacaccacttctacttactttggaactcaaggtttgttccacctctccaatcaacattttttaaatcactctgatttactagtctaattacatcataatatatacaaaacataaaataacagatttaatagttttgttttctaactattttacgttttcttttaaatgtgtataaactttaggcccgacgatgttactctacacattccccgtcttgttcatggccgtagtgggaagtgtatatctccatttaagaaaaaaggcgaatcaaaaccgagatgaagggtatatatatatataatagttttttacttatttcagtaaattaaataactgtttatttttactttatactatttcatgatggttaaatatatctttcctttctcaaattttagagaaaaagaagctacacccgataacttgagtatatggagaagaccaatgatcatcaaaggtctcgggatcgtctcgaaaatcgagctcgctttctttgttatgtttatcgctcttatcgtctggtctttcacgacatacttacacgtcggttttgccaaaatcaatcataaaacagcggcaaaaaagggagaggaagtgtaagtgaatcaatattttaaatattttgcaaatactacattcgtatattattattaacccgcgatcgattcttttggttgatagttgggaatcaaagcttgattcggtggctctacggttcggattaattggcaacttgtgtctagcatttctgttcttcccggtgactcgaggatcgtctatattgtcgttgttcgggcttacttctgaggcgagtatcaagtatcacatatggctcggtcatattgttatgactctattcacttctcatggtgtttgttacattatttattggatcgttaccaaacagacacatgaggtaccttaatttttatattattatttatgaattataaattagttaatatttatggctcacaattcctgaaaatattctgccagtgaatttggaaaactgaagataaagtccataaatgttagaagattttccactttgaattaaagtcaacttatataatggtcccaaatcatcgaacattgtaaaaattaactcaccaatgtgaaaaaccgaagataggatcatatcccataactttattctttggtgatgaaatgacgaagctaacataatttatttaacagtcccttttaaaaatttctgatagatgttagacgtaattaattagttaattaattattactcaccgaacaatgacaaatgcttataaaagttgtttttgaactatcgttgttgatccgttgatgtcttttttcatatatgatatccaattttcctagtagtgtattaaataatgctatatgtttttttagatgttgaaatgggaaaaaatcggcatatcaaatgtagccggagagttggctttggtagccggattgattatgtgggcaacaacgtttccaaggattagacgaaagatgtttgaagttttcttctacgcacatcacttatacatccaatttatcgtgttcttcgtgttccatgttggcatagcatatgcatccatcatgctaccgggattctacctcttcatgattgatcgaatcttgagatttttacaatcaaagggaaacgttcgtgtggtttctgctcgtgttcttccgtgtgaatctctcgagctcaacttctccaaaagccaaggtacgtaaaatagagcacaaaaagtatagaaaatataaaggatcaatttctttttaagtgataatggtcgttaacatttgtcttttaattttaagtcttttagatgtcacaattttcatttttttatataggtctacaatatacaccaacaagcatcatattcatcaatgtcccaagcatttcaaaggctcaatggcatccattcaccattacttctagtagcaatttggagcccgaaaagctaagtgttatgatcaaaagtgaaggaagttggtctaggaaactttaccaaatgttatcatccccaaattctattgaccggcttgatgtatgcattgaaggaccttatgggcctatttcaaccaactttctaaggtattatgttcattacaatgacttgtgttaggttcatttcattttattatacttaaaatgatcaaattatggtttcaggcacgatatgctagtgatggtgagcggaggaagtgggataacaccatttatctcaatatttagggagcttgtttacactaccgaaaccctaaaacgtaaagctccaaaaattctcttgataagttcgtttaaagactcttctgatctcaccatgctagaattgttattaccatcatctggtgcacctatagagttttcaaaactagagttacaaatcgaggcatatgtgacaagagaaaaccagcccgttaatgataagaaactagtgactgccttatggtttaaaccaaatccctctgacgcacccatcactcctattttaggacaaaatggttggttatggcttggtgcgattattgcatgttcttttgtgattttccttgtatctatggggcttgtaacacggttttacatctatcctattgataataacaccaacaaggtgtattcatatggatcgagggccgtgttaaacatgttgctcatttgtgtgtctataatggtaacatgttgtttcggattttggtggaataaaaagagaaacgctatggactcaaagcaaattcaaagcatggagggtgtgacacccgttagctcacccaactcatggttttataacgcggatagagagcttgaaagtgttccccaacaatcgctctttcagtctacaaatgttcattttggcaaaagaccggatcttaagagtaagaccagattctatgtctaatgctacaaaagttacacacttttgaatatatgttaatacaaaccctaacactttctattttgtttatatttttgttaggaattttgtttgagcaaaaagaatcaagtgttggagttcttgtttgtgggccaaaaaagatgaggcatgaggctgcaaatatatgttcatccggattggcttcaaacttgcattttgagtccataagttttagttggtga

SEQ ID NO: 23 - DNA, 2850 bp, Arabidopsis thaliana
  CDS (167)..(2578)
aaatattgttaccataaattcataaactttcgttaaacttaaagtgatttatacacatagtatattcaaatatcgataaatgtattttgctaatcaaatcgtatattcttttataccagttttttaacgtcatctcgccaaaacaacaacaaatagatgtaaaataatgaaagaaaacaaaaaacaagatccatggggaagagtcacatgcatggagcatgcaactagcttacttcatccaattcccactcaaaattctctctttatatatacactttctctaccactacttccctcaaaacaagctaactcgatccttctcactaaagcgatcgtaccgatcttaatatctttagcgagcgagagagagagagatagaaatcctgagaggaaagagaggatggagatcgaaaaaagcaataacggtggttcgaacccatctgcaggagaagaatttaaggatatgattaagggagtgactaagttcttgatgatggtgattttccttggaaccatcatgctttggatcatgatgccaacactaacctatcgaaccaagtggttgccacatctgcgtatcaagtttggaacatccacttattttggtgccacagggacgacgcttttcatgtatatgttcccaatgatggtcgtagcttgtttgggatgtgtctatcttcacttcaagaatcgaaagtcgccacaccatatcgatagggagacgaagggaggagtgtggagtaaactaagaaagccaatgttagtgaaggggccattaggaatagtctcagtgactgagatcaccttcttggcgatgtttgtggctcttcttctctggtgctttatcacttatttgcgcaatagcttcgccactatcactcctaaatcagctgccgcacatgacgaatctttgtggcaagcgaagctggaatcagcggcgctaaggttaggactgatcggaaacatatgtttggcgttcttgttcttaccggtggctcgtgggtcatcgttgctaccggcaatgggattaacctcggagtcaagcatcaaataccatatatggctcggccacatggtcatggcccttttcaccgttcatggtctttgttacataatttactgggcctcaatgcatgaaatctcccagatgatcatgtgggatacgaaaggtgtctcaaatttggccggagagatagctctggcggccggacttgtgatgtgggccaccacatatccgaagataaggagaagattcttcgaagtcttcttctacactcactatctctacatcgtcttcatgctcttctttgtcctccacgtcggcataagtttctccttcatcgctctccctggtttctacatcttcttagtcgatcgtttccttcggtttcttcagtcacgtgaaaatgttcgcttgctcgctgctcggattcttccttccgacactatggagctcactttctccaaaaactctaagttggtttatagcccgacgagcataatgtttgtgaacataccgagcatttcaaagctgcaatggcatccgtttacgataacttccagtagcaaactcgaaccagagaagctaagtattgttatcaagaaagaaggcaaatggtcaactaagcttcaccagaggctttcttcttctgatcagatcgaccgacttgctgtttctgtagaaggtccttacggccctgcttccgccgatttcttaaggcatgaagctttggttatggtgtgcggaggaagcgggataactccgtttatctctgttattcgtgatttgatcgccacaagccaaaaggaaacatgcaaaatcccaaaaataactctcatttgtgcgtttaagaagtcttcagagatctccatgctcgatcttgtcttgccattatccggtcttgagactgaactatcctccgacattaacatcaaaatcgaagccttcataacccgagataatgatgcaggagatgaagcaaaagctgggaaaatcaaaactctctggttcaaaccaagtctttcagaccaatccatctcatcaatcctcggaccaaactcatggctttggctcggtgcaattctcgcatcttcgttcttgatcttcatgataattattggtatcatcactaggtattacatttacccgatcgaccacaacaccaacaagatctattctttgacttcaaaaaccatcatatatatcttggtcatctccgtgagcataatggcgacttgtagtgcggctatgttgtggaacaagaagaagtatggtaaagttgaaagtaaacaggtccaaaacgtcgaccgtccatctccaacatcttctcctacctcatcatggggttacaattccttgagagaaatcgaaagtacgccacaagaatcgctcgtgcaacgcaccaatctgcattttggagaaagacctaatctcaagaaacttctacttgatgtggaaggttcgagtgtgggagttcttgtttgtggtcctaagaagatgagacaaaaggttgcggaaatatgttcctctggtttggctgagaatcttcattttgaatctatcagtttcagctggtgattgcgtatataactctgttttcactatgtgttgtgcaatttgcttgagttgcaagttaataaggtggccctgtgatttgacctatctttgtgtgctttacattgacttttcctgttttttgtttttctttatcctcttctaggaatattcagtgttaaaaaaaaaacttcctttcaaaagttccggaatatcctttttttgtttgtaacacaaggcatacagcttttgtaaattgtaaatgttgaaatataatactcatgttgggtcatata

SEQ ID NO: 24 - protein, 803 aa, Arabidopsis thaliana
MKENKKQDPWGRVTCMEHATSLLHPIPTQNSLFIYTLSLPLLPSKQANSILLTKAIVPILISLASERERDRNPERKERMEIEKSNNGGSNPSAGEEFKDMIKGVTKFLMMVIFLGTIMLWIMMPTLTYRTKWLPHLRIKFGTSTYFGATGTTLFMYMFPMMVVACLGCVYLHFKNRKSPHHIDRETKGGVWSKLRKPMLVKGPLGIVSVTEITFLAMFVALLLWCFITYLRNSFATITPKSAAAHDESLWQAKLESAALRLGLIGNICLAFLFLPVARGSSLLPAMGLTSESSIKYHIWLGHMVMALFTVHGLCYIIYWASMHEISQMIMWDTKGVSNLAGEIALAAGLVMWATTYPKIRRRFFEVFFYTHYLYIVFMLFFVLHVGISFSFIALPGFYIFLVDRFLRFLQSRENVRLLAARILPSDTMELTFSKNSKLVYSPTSIMFVNIPSISKLQWHPFTITSSSKLEPEKLSIVIKKEGKWSTKLHQRLSSSDQIDRLAVSVEGPYGPASADFLRHEALVMVCGGSGITPFISVIRDLIATSQKETCKIPKITLICAFKKSSEISMLDLVLPLSGLETELSSDINIKIEAFITRDNDAGDEAKAGKIKTLWFKPSLSDQSISSILGPNSWLWLGAILASSFLIFMIIIGIITRYYIYPIDHNTNKIYSLTSKTIIYILVISVSIMATCSAAMLWNKKKYGKVESKQVQNVDRPSPTSSPTSSWGYNSLREIESTPQESLVQRTNLHFGERPNLKKLLLDVEGSSVGVLVCGPKKMRQKVAEICSSGLAENLHFESISFSW

SEQ ID NO: 25 - DNA, 2374 bp, Medicago truncatula
  CDS (64)..(2214)
gtttcttcttctctctaaacaattaaattttcacacacaaccgagaagaaacaacaacaaaaaatggctcaagataaagtgaaaaggtcacctactcaaataaaatatggattaattcaatctacaataaggttattgatggtgttactgtttctgggtttaattttcatttttataatgatgcctacatatactttcaaacacacatggaatcctcaattccaagcaaagactaattctacatattttggtgcacaaggtacaaggattcttatttacacttttccagtgttgttaatagccactttgggatgtgtctttctccacatagccaaaaaatcaaatgagagcaacatggaaattggcaatgggaagaaacatgggacaaccatatggaatcgtccaatgcttgtgaaaggacctcttggaattgtttctattacagaaatagcattcttgcttatgttcattgcacttctaatttggtccttttccatttatttacacaacgactttgcaacaatcatatcaaaatcagaggcagagaatggcgaaaaagtgtggcaagagaaaatagaaagtgtggcactaaggttaggtcttgttggtaacatatgtttggcattgttatttttcccagtgactcgtggatcaaccgtgctaccaatatttggcctcacttctgaaggttgcatcaaataccacatttggcttgggcacgtgcttatgacacttttcactactcatggagtttgttacattatctattgggcatctactcatcaaatttcacagatgctgaaatgggacaaagttggagtatcaaatgtggctggagagatatctttgcttgctggtttagtcttatgggttgcaaccattccttacattaggagaaaatactttgagctatttttctacactcattacctctacattatcttcatcatcttcttcatctttcatgttggcatttcctttgcctgcattatgctccctggtttctacctcttcttggttgatcgttacctacggttcctacaatctaggcgcgaagttcgtttggtttcatctcgtgttttgccgtgtgaaactgtagaactcaacttctctaagggacatggattgacgtataatccaacaagtgtgatgttcataaatgtaccaagcatatcaaagttgcaatggcatccatttaccattacttctaatagtaaattggaatctgaaaagctaagtgttgtcattaaaagtgaaggaacttggacaaaaaagctctaccagttgctttcaaatccttcgcctatcgatcgccttggaatatctgttgaaggtccttatggacctgcttcaaccaattatctaaggcatgacacacttgtgatggtgagtggaggaagtggcatcacaccatttatctctatcattagagagctaatatatcttagcactacattcaaatgcaagacaccaaacattgtcctaatttcttcattcaagaatacttcatgtttgtcaatgctagatttgatcctacctatttctggcacaccatctgacatttctaatattcaactccaaattgaggcatacatcacaagagacagagagtttaaatcagatagctcaattcatcctcaaactttatggtttaagccaaatccaacagatgcaccaatacattctatgttaggtccaaacacttggctttggcttggtgctataatctcatcttctttcattatcttccttatcataatcgggatcattactcgatactacattttcccgattgatcataacacgaataaaatattctcgtatcctttaagggtgttccttaacgtgctagtaatatgtgtgtcggtagttgttgttgctagtgtagcagttatttggaataaaaaacaaaatgctaaagaagcaaaacagattcagaacttggaagggtcatcaccaacagtgtcaccaagttcaatgatttacaatgttgatagagaattagaaagccttccatatcagtccctagttcaagctaccaatgtgcattatggaacaagacctgatcttaaaagacttctatttgaaatgaaagggtcaagtgtgggagttcttgtttcaggacctaaacaaatgaggcaggaggttgcatccatttgttcatctggtttagttgaaaatctgcattttgagtccataagttttacctggtgattttattcattctaattcaaagggtgcaaaccatccatgatcaatctctatagtaggacttcattttaattgccttgattaaaaaatctgtaaaatttgtttttcaacaaataactaggctttcttgtataccatatatgacatgaatgaagtttaatga

SEQ ID NO: 26 - protein, 716 aa, Medicago truncatula
MAQDKVKRSPTQIKYGLIQSTIRLLMVLLFLGLIFIFIMMPTYTFKHTWNPQFQAKTNSTYFGAQGTRILIYTFPVLLIATLGCVFLHIAKKSNESNMEIGNGKKHGTTIWNRPMLVKGPLGIVSITEIAFLLMFIALLIWSFSIYLHNDFATIISKSEAENGEKVWQEKIESVALRLGLVGNICLALLFFPVTRGSTVLPIFGLTSEGCIKYHIWLGHVLMTLFTTHGVCYIIYWASTHQISQMLKWDKVGVSNVAGEISLLAGLVLWVATIPYIRRKYFELFFYTHYLYIIFIIFFIFHVGISFACIMLPGFYLFLVDRYLRFLQSRREVRLVSSRVLPCETVELNFSKGHGLTYNPTSVMFINVPSISKLQWHPFTITSNSKLESEKLSVVIKSEGTWTKKLYQLLSNPSPIDRLGISVEGPYGPASTNYLRHDTLVMVSGGSGITPFISIIRELIYLSTTFKCKTPNIVLISSFKNTSCLSMLDLILPISGTPSDISNIQLQIEAYITRDREFKSDSSIHPQTLWFKPNPTDAPIHSMLGPNTWLWLGAIISSSFIIFLIIIGIITRYYIFPIDHNTNKIFSYPLRVFLNVLVICVSVVVVASVAVIWNKKQNAKEAKQIQNLEGSSPTVSPSSMIYNVDRELESLPYQSLVQATNVHYGTRPDLKRLLFEMKGSSVGVLVSGPKQMRQEVASICSSGLVENLHFESISFTW

SEQ ID NO: 27 - DNA, 2406 bp, Helianthus annuus
  CDS (54)..(2162)
cttttacaaaccaactagagagagaaatatcaaagatatatagtaagaagaagatgatgatgcttatgaagatgatcaaagggcttgcaatgatggtcttcataggctatcttttcctatgggtgatcacaccaacctatgtttttaagaaaaagtggatccttagggttcgagcccacaccacttctacttactttggaactcaaggtccaacgatgttgctctacacattgcccgttttgatcatggccgtcttgggaagtgtgtatctccatttaagaaaaaaggcgaaccaaaaccgcgacgaaggagataaagaagctacttccgataacttgagtatatggaaaaggccaatgatcatcaaaggtctcggaatcgtctcgataatcgagctcgctttcttcgttatgtttatcgctctcattgtctggtctttcacaacatacttacatgtcagttttgccggtattaaccataaaacagcagcaaaaaatggagaagaagtttggcaatcaaagttgagttcagtggctctacggttcgggttaattggtaacttgtgtctagtatttttgttcttcccagtgactcgaggatcgtctatattgtcgctgttcgggctaacttctgaggccagcatcaagtatcacatatggctgggccatattgttatgaccctcttcacttctcatggtgtttgttacattatttattggatagtaaccaagcagacatcagagatggtgaaatgggcaaaaaccgacatatcaaatgtagccggagagttggctttggtagcaggattgattatgtgggcaacgacgtttcctaggattagacgaaagatgtttgaggttttcttctacacgcatcacttgtacatcctatttgtcgtgttcttcgtgttccatgttggcatagcatatgcctccatgatgcttcctggattctaccttttcatgattgatcggtacttgagatttttacaatcaaaagggaaggttcgtttggtttcttcgcgtgttcttccatgtgaaactctcgagctcaacttctccaagagccgaggtttgaattatacaccaacaagcatcatattcatcaatatcccaagcatttcaaaggctcaatggcatccattcaccattacttcaagtagcaatttggagcctgaaaagctaagtgttatgatcaaaagtgaagggagttggtctaggaaactctaccaaatgttatcatccccgaattctatagatcggcttgatgtgtgcgttgaaggaccttatggacccgttgcaaccaattttctaaggcacgatatgctagtgatggtgagcggaggaagtgggataacaccgtttatctcgatatttagggagcttgtttacacaaccgaaaccctaaaatgtaaagctccaaaaattctcttgataagtgcgtttaaaaactcatctgatcttaccatgctagaattgttattaccatcatccggttcacctatagagttttcaaaactagagttacaaatcgaggcctatgtaacaagagagaaacaacccgtgaccgatgataagaaactagtgaataccctttggcttaaaccaaacccctccgatgcgcacataactcctgttttaggacaaaatggttggttatggcttggcgcaattattgtatcttcttttgtggttttccttgtgtctatgggacttgtaacgcgcttttacatctatcctattgataagaacacaaacaaagtgtactcactaggatcgagggccgcgttaaatatgttgctcatttgtgtgtcgattatggtaacatgttatatgggtttttggtggaataagaagagaaatgctatggattcaaagcaaattcaaaacatggagggggcgacacccgttaactcacccaactcatggttttataacgcggatagagagcttgaaagcatgcctcaacaatcactttatcagtctacaaatgtgcattttggcaaaaggccggatcttaagagaattatgtttgagcaaaaagaatcaagtgttggagttctagtttgtgggccaaagaaaatgaggcatgaggttgcaaacatatgttcatctggattggcttcaaacttgcattttgagtccataagctttagctggtgatcgactggtcggcttttgcaaattgcaaaacatggtgtgcgacgagttggtttttcttttcatattcgtcacttacaagttttgatgattcaaagttcaaggtttcagttttgttccgatagagcgtccaaaatatagaaatgtgtgtaaatcggatacaagggtgccttatctttccttttgcttgtaaacttgtaatgcataaataaactgtttatatatcaaactttttgtatttaaatta

SEQ ID NO: 28 - protein, 702 aa, Helianthus annuus
MMMLMKMIKGLAMMVFIGYLFLWVITPTYVFKKKWILRVRAHTTSTYFGTQGPTMLLYTLPVLIMAVLGSVYLHLRKKANQNRDEGDKEATSDNLSIWKRPMIIKGLGIVSIIELAFFVMFIALIVWSFTTYLHVSFAGINHKTAAKNGEEVWQSKLSSVALRFGLIGNLCLVFLFFPVTRGSSILSLFGLTSEASIKYHIWLGHIVMTLFTSHGVCYIIYWIVTKQTSEMVKWAKTDISNVAGELALVAGLIMWATTFPRIRRKMFEVFFYTHHLYILFVVFFVFHVGIAYASMMLPGFYLFMIDRYLRFLQSKGKVRLVSSRVLPCETLELNFSKSRGLNYTPTSIIFINIPSISKAQWHPFTITSSSNLEPEKLSVMIKSEGSWSRKLYQMLSSPNSIDRLDVCVEGPYGPVATNFLRHDMLVMVSGGSGITPFISIFRELVYTTETLKCKAPKILLISAFKNSSDLTMLELLLPSSGSPIEFSKLELQIEAYVTREKQPVTDDKKLVNTLWLKPNPSDAHITPVLGQNGWLWLGAIIVSSFVVFLVSMGLVTRFYIYPIDKNTNKVYSLGSRAALNMLLICVSIMVTCYMGFWWNKKRNAMDSKQIQNMEGATPVNSPNSWFYNADRELESMPQQSLYQSTNVHFGKRPDLKRIMFEQKESSVGVLVCGPKKMRHEVANICSSGLASNLHFESISFSW

SEQ ID NO: 29 - DNA, 2254 bp, Manihot esculenta
  CDS (1)..(2244)
atggattcagaatcagcttctaacacagaaagtaaccatatggttcggacagggattaagacaacattgtgggtagtactgggaggatatgctgtgttttgggttatgatgcccactaatacctaccaacaaacatggcgttcttatttgagagttcatatcgattccacctactttgggactcaagctaatatgtttccttgtatttcttcccttgctttcgtttcaatgactggttttattttacggctatgggggctttctgcttatgcatgtaaacttgtttcaggtccaaaccttttggtacatttcgccaccattcttttcattgctttgctgggttgtgtttatctccatgtagtaaagagatcaaatcacagtaacttcgaaaggtacaatggcagaaaacaactcttggccacatggaagaagccgatgctagtgaaaggccctctgggaatcgtttctggaatagagctggccttcttgatcatgtttgttgcactgttggtttggtctttatcaacctatttgcatgacagcttttctaccatcaccccacagtcggctgcagggagtggggagactgtatgggaagctaaaatggagaacgcagcccttaggctagggttggtggggaacatatgtctgacgttgctcttcttcccggtgactcgagggtcatcgattctgccattgtttgggctcacctcagagggtagcattaagtaccacatatggcttggtcacactgtgatggctttcttcaccgcacatggagtttgttacatcatctattgggctgctaccgatcagatttccgagatgctgaaatgggcaaaggttgggatatcaaatgtggctggggagattgctttgcttgctgggctgggcctgtgggctacaaccttcactcgcataagaagaaaaatgtttgagctcttcttttacactcatcatctctacatcctcttcatgattttctatgtattacatgttcccatctcttttgcctgtattacaatccctggattttacctcttcttggtcgatcgttttctgaggttcttacaatcacgacaaagagttcgtgctgtctcatcccgcattctgccttgcgaaactttagaaatcaacttctccaaaaaccctggtttgagtttcaatccaacgagcatcctgtttataaatgtgcctagcatttctaagctgcaatggcatcctttcacaatcacttctaatagtaacttagaacctgagatgctgagtgttatgattaaaagtgaaggaagttggtccaggaagctgcatcagatgctttcatctccttcctcaattgatcgtcttgaagtttcagttgaaggaccttatggacctgcttcaactcactttctaaggcatgacacacttgtgatggtgagtggaggcagtggcattactccttttatatctataattcgagaactcatctttgcttccacaacatacaaatcaaagattccacaagtactcctaatttgctcattcaagaactcttcagacctgaccatgctagatctcctacttccaatatctggcaccccatcagaaatttccagtctgcagctaaaaatcgaggcttatgttacgagagagaaagaaccctcaaccagcaacgggaagctccttcgaactctatggttcaagccccacccaacagataaacctgtttctgccattttaggccccaaaagctggctatggcttggcgcgataatatcatcttcgtttatcattttcctcatcataattggccttattacccgctattacatttatcctatcgatcataacacctccagtattttctcatactctttccgatcttttcttaatatgttagtaatatgcatatgcatagccataacagcaagtgcagcctttttatggaacaagaaaataaatggaaagcaaccgaatcagattcagaacattgaagggtccacaccaaatacatcaccaggctcatgggtatatgatggtgggagagaattggaaagtcttccacatcagtctcttgtccaggctactaatgtgcactatggcgaaagacctgatctgaagagaacactacttgattgcaaaggatcaagtgtgggggttcttgtttgtggtccgaagcagatgaggcatgagattgcaatgatatgttcatctggattggcagataacttgcactttgagtccattagctttagctggtgatctagtcatc

SEQ ID NO: 30 - protein, 747 aa, Manihot esculenta
MDSESASNTESNHMVRTGIKTTLWVVLGGYAVFWVMMPTNTYQQTWRSYLRVHIDSTYFGTQANMFPCISSLAFVSMTGFILRLWGLSAYACKLVSGPNLLVHFATILFIALLGCVYLHVVKRSNHSNFERYNGRKQLLATWKKPMLVKGPLGIVSGIELAFLIMFVALLVWSLSTYLHDSFSTITPQSAAGSGETVWEAKMENAALRLGLVGNICLTLLFFPVTRGSSILPLFGLTSEGSIKYHIWLGHTVMAFFTAHGVCYIIYWAATDQISEMLKWAKVGISNVAGEIALLAGLGLWATTFTRIRRKMFELFFYTHHLYILFMIFYVLHVPISFACITIPGFYLFLVDRFLRFLQSRQRVRAVSSRILPCETLEINFSKNPGLSFNPTSILFINVPSISKLQWHPFTITSNSNLEPEMLSVMIKSEGSWSRKLHQMLSSPSSIDRLEVSVEGPYGPASTHFLRHDTLVMVSGGSGITPFISIIRELIFASTTYKSKIPQVLLICSFKNSSDLTMLDLLLPISGTPSEISSLQLKIEAYVTREKEPSTSNGKLLRTLWFKPHPTDKPVSAILGPKSWLWLGAIISSSFIIFLIIIGLITRYYIYPIDHNTSSIFSYSFRSFLNMLVICICIAITASAAFLWNKKINGKQPNQIQNIEGSTPNTSPGSWVYDGGRELESLPHQSLVQATNVHYGERPDLKRTLLDCKGSSVGVLVCGPKQMRHEIAMICSSGLADNLHFESISFSW